European Patent Specification EP 3 505 538 B1, published May 1, 2024. Title: Method for Production of Antigen Fusion Proteins. Applicant: JCR Pharmaceuticals Co., Ltd. The sequence listing filed with the application follows.

SEQUENCE LISTING (28 sequences)

SEQ ID NO: 1 - protein, 5 aa, Artificial Sequence
  Amino acid sequence of an exemplified linker 1
GGGGS

SEQ ID NO: 2 - protein, 6 aa, Artificial Sequence
  Amino acid sequence of an exemplified linker 2
GGGGGS

SEQ ID NO: 3 - protein, 6 aa, Artificial Sequence
  Amino acid sequence of an exemplified linker 3
SGGGGG

SEQ ID NO: 4 - protein, 760 aa, Homo sapiens
MMDQARSAFSNLFGGEPLSYTRFSLARQVDGDNSHVEMKLAVDEEENADNNTKANVTKPKRCSGSICYGTIAVIVFFLIGFMIGYLGYCKGVEPKTECERLAGTESPVREEPGEDFPAARRLYWDDLKRKLSEKLDSTDFTGTIKLLNENSYVPREAGSQKDENLALYVENQFREFKLSKVWRDQHFVKIQVKDSAQNSVIIVDKNGRLVYLVENPGGYVAYSKAATVTGKLVHANFGTKKDFEDLYTPVNGSIVIVRAGKITFAEKVANAESLNAIGVLIYMDQTKFPIVNAELSFFGHAHLGTGDPYTPGFPSFNHTQFPPSRSSGLPNIPVQTISRAAAEKLFGNMEGDCPSDWKTDSTCRMVTSESKNVKLTVSNVLKEIKILNIFGVIKGFVEPDHYVVVGAQRDAWGPGAAKSGVGTALLLKLAQMFSDMVLKDGFQPSRSIIFASWSAGDFGSVGATEWLEGYLSSLHLKAFTYINLDKAVLGTSNFKVSASPLLYTLIEKTMQNVKHPVTGQFLYQDSNWASKVEKLTLDNAAFPFLAYSGIPAVSFCFCEDTDYPYLGTTMDTYKELIERIPELNKVARAAAEVAGQFVIKLTHDVELNLDYERYNSQLLSFVRDLNQYRADIKEMGLSLQWLYSARGDFFRATSRLTTDFGNAEKTDRFVMKKLNDRVMRVEYHFLSPYVSPKESPFRHVFWGSGSHTLPALLENLKLRKQNNGAFNETLFRNQLALATWTIQGAANALSGDVWDIDNEF

SEQ ID NO: 5 - protein, 525 aa, Homo sapiens
SETQANSTTDALNVLLIIVDDLRPSLGCYGDKLVRSPNIDQLASHSLLFQNAFAQQAVCAPSRVSFLTGRRPDTTRLYDFNSYWRVHAGNFSTIPQYFKENGYVTMSVGKVFHPGISSNHTDDSPYSWSFPPYHPSSEKYENTKTCRGPDGELHANLLCPVDVLDVPEGTLPDKQSTEQAIQLLEKMKTSASPFFLAVGYHKPHIPFRYPKEFQKLYPLENITLAPDPEVPDGLPPVAYNPWMDIRQREDVQALNISVPYGPIPVDFQRKIRQSYFASVSYLDTQVGRLLSALDDLQLANSTIIAFTSDHGWALGEHGEWAKYSNFDVATHVPLIFYVPGRTASLPEAGEKLFPYLDPFDSASQLMEPGRQSMDLVELVSLFPTLAGLAGLQVPPRCPVPSFHVELCREGKNLLKHFRFRDLEEDPYLPGNPRELIAYSQYPRPSDIPQWNSDKPSLKDIKIMGYSIRTIDYRYTVWVGFNPDEFLANFSDIHAGELYFVDSDPLQDHNMYNDSQGGDLFQLLMP

SEQ ID NO: 6 - protein, 214 aa, Artificial Sequence
  Amino acid sequence of the light-chain of humanized anti-hTfR antibody No.1
DIQVTQSPSFLSASVGDRVTITCKASQDVNSAVAWFQQKPGKAPKLLIYWTSTRHTGVPDRFSGSGSGTVYTLTISSLQPEDFATYYCQQHYSTPRTFGGGTKVEIKRTVAAPSVFIFPPSDEQLKSGTASVVCLLNNFYPREAKVQWKVDNALQSGNSQESVTEQDSKDSTYSLSSTLTLSKADYEKHKVYACEVTHQGLSSPVTKSFNRGEC

SEQ ID NO: 7 - protein, 446 aa, Artificial Sequence
  Amino acid sequence of the heavy-chain of humanized anti-hTfR antibody No.1
EVQLVESGGGLVQPGGSLRLSCAASGLTFSNYGMSWVRQAPGKGLELVANINTNGGSTYYPDSVKGRFTISRDNAKNSLYLQMNSLRAEDTAVYYCTNNRYDEDYWGQGTLVTVSSASTKGPSVFPLAPSSKSTSGGTAALGCLVKDYFPEPVTVSWNSGALTSGVHTFPAVLQSSGLYSLSSVVTVPSSSLGTQTYICNVNHKPSNTKVDKKVEPKSCDKTHTCPPCPAPELLGGPSVFLFPPKPKDTLMISRTPEVTCVVVDVSHEDPEVKFNWYVDGVEVHNAKTKPREEQYNSTYRVVSVLTVLHQDWLNGKEYKCKVSNKALPAPIEKTISKAKGQPREPQVYTLPPSRDELTKNQVSLTCLVKGFYPSDIAVEWESNGQPENNYKTTPPVLDSDGSFFLYSKLTVDKSRWQQGNVFSCSVMHEALHNHYTQKSLSLSPGK

SEQ ID NO: 8 - protein, 214 aa, Artificial Sequence
  Amino acid sequence of the light-chain of humanized anti-hTfR antibody No.2
EIVLTQSPDFQSVTPKEKVTITCRASQSISNNLQWYQQKPDQSPKLLIKYASQSISGIPSRFSGSGSGTDFTLTINSLEAEDAATYLCQQSNSWPRTFGQGTKVEIKRTVAAPSVFIFPPSDEQLKSGTASVVCLLNNFYPREAKVQWKVDNALQSGNSQESVTEQDSKDSTYSLSSTLTLSKADYEKHKVYACEVTHQGLSSPVTKSFNRGEC

SEQ ID NO: 9 - protein, 453 aa, Artificial Sequence
  Amino acid sequence of the heavy-chain of humanized anti-hTfR antibody No.2
QVQLVQSGAEVKKPGASVKVSCKASGYTFTDYVMHWVRQAPGQGLEWIGVISTYYGHGSYNQRFKGRATMTVDKSISTAYMELVRLRSDDTAVYYCVRGGYGSSSLAGNFDVWGQGTTVTVSSASTKGPSVFPLAPSSKSTSGGTAALGCLVKDYFPEPVTVSWNSGALTSGVHTFPAVLQSSGLYSLSSVVTVPSSSLGTQTYICNVNHKPSNTKVDKKVEPKSCDKTHTCPPCPAPELLGGPSVFLFPPKPKDTLMISRTPEVTCVVVDVSHEDPEVKFNWYVDGVEVHNAKTKPREEQYNSTYRVVSVLTVLHQDWLNGKEYKCKVSNKALPAPIEKTISKAKGQPREPQVYTLPPSRDELTKNQVSLTCLVKGFYPSDIAVEWESNGQPENNYKTTPPVLDSDGSFFLYSKLTVDKSRWQQGNVFSCSVMHEALHNHYTQKSLSLSPGK

SEQ ID NO: 10 - protein, 219 aa, Artificial Sequence
  Amino acid sequence of the light-chain of humanized anti-hTfR antibody No.3
DIVMTQTPLSLSVTPGQPASISCRSSQSLVHSNGNTYLHWYLQKPGQSPQLLIYKVSNRFSGVPDRFSGSGSGTDFTLKISRVEAEDVGVYYCSQSTHVPWTFGQGTKVEIKRTVAAPSVFIFPPSDEQLKSGTASVVCLLNNFYPREAKVQWKVDNALQSGNSQESVTEQDSKDSTYSLSSTLTLSKADYEKHKVYACEVTHQGLSSPVTKSFNRGEC

SEQ ID NO: 11 - protein, 448 aa, Artificial Sequence
  amino acid sequence of the heavy-chain of humanized anti-hTfR antibody No.3
EVQLVQSGAEVKKPGESLKISCKGSGYSFTNYWLGWVRQMPGKGLEWMGDIYPGGDYPTYSEKFKVQVTISADKSISTAYLQWSSLKASDTAMYYCARSGNYDEVAYWGQGTLVTVSSASTKGPSVFPLAPSSKSTSGGTAALGCLVKDYFPEPVTVSWNSGALTSGVHTFPAVLQSSGLYSLSSVVTVPSSSLGTQTYICNVNHKPSNTKVDKKVEPKSCDKTHTCPPCPAPELLGGPSVFLFPPKPKDTLMISRTPEVTCVVVDVSHEDPEVKFNWYVDGVEVHNAKTKPREEQYNSTYRVVSVLTVLHQDWLNGKEYKCKVSNKALPAPIEKTISKAKGQPREPQVYTLPPSRDELTKNQVSLTCLVKGFYPSDIAVEWESNGQPENNYKTTPPVLDSDGSFFLYSKLTVDKSRWQQGNVFSCSVMHEALHNHYTQKSLSLSPGK

SEQ ID NO: 12 - protein, 973 aa, Artificial Sequence
  Amino acid sequence of fusion protein of the heavy-chain of humanized anti-hTfR antibody No.1 and hI2S
EVQLVESGGGLVQPGGSLRLSCAASGLTFSNYGMSWVRQAPGKGLELVANINTNGGSTYYPDSVKGRFTISRDNAKNSLYLQMNSLRAEDTAVYYCTNNRYDEDYWGQGTLVTVSSASTKGPSVFPLAPSSKSTSGGTAALGCLVKDYFPEPVTVSWNSGALTSGVHTFPAVLQSSGLYSLSSVVTVPSSSLGTQTYICNVNHKPSNTKVDKKVEPKSCDKTHTCPPCPAPELLGGPSVFLFPPKPKDTLMISRTPEVTCVVVDVSHEDPEVKFNWYVDGVEVHNAKTKPREEQYNSTYRVVSVLTVLHQDWLNGKEYKCKVSNKALPAPIEKTISKAKGQPREPQVYTLPPSRDELTKNQVSLTCLVKGFYPSDIAVEWESNGQPENNYKTTPPVLDSDGSFFLYSKLTVDKSRWQQGNVFSCSVMHEALHNHYTQKSLSLSPGKGSSETQANSTTDALNVLLIIVDDLRPSLGCYGDKLVRSPNIDQLASHSLLFQNAFAQQAVCAPSRVSFLTGRRPDTTRLYDFNSYWRVHAGNFSTIPQYFKENGYVTMSVGKVFHPGISSNHTDDSPYSWSFPPYHPSSEKYENTKTCRGPDGELHANLLCPVDVLDVPEGTLPDKQSTEQAIQLLEKMKTSASPFFLAVGYHKPHIPFRYPKEFQKLYPLENITLAPDPEVPDGLPPVAYNPWMDIRQREDVQALNISVPYGPIPVDFQRKIRQSYFASVSYLDTQVGRLLSALDDLQLANSTIIAFTSDHGWALGEHGEWAKYSNFDVATHVPLIFYVPGRTASLPEAGEKLFPYLDPFDSASQLMEPGRQSMDLVELVSLFPTLAGLAGLQVPPRCPVPSFHVELCREGKNLLKHFRFRDLEEDPYLPGNPRELIAYSQYPRPSDIPQWNSDKPSLKDIKIMGYSIRTIDYRYTVWVGFNPDEFLANFSDIHAGELYFVDSDPLQDHNMYNDSQGGDLFQLLMP

SEQ ID NO: 13 - protein, 980 aa, Artificial Sequence
  Amino acid sequence of fusion protein of the heavy-chain of humanized anti-hTfR antibody No.2 and hI2S
QVQLVQSGAEVKKPGASVKVSCKASGYTFTDYVMHWVRQAPGQGLEWIGVISTYYGHGSYNQRFKGRATMTVDKSISTAYMELVRLRSDDTAVYYCVRGGYGSSSLAGNFDVWGQGTTVTVSSASTKGPSVFPLAPSSKSTSGGTAALGCLVKDYFPEPVTVSWNSGALTSGVHTFPAVLQSSGLYSLSSVVTVPSSSLGTQTYICNVNHKPSNTKVDKKVEPKSCDKTHTCPPCPAPELLGGPSVFLFPPKPKDTLMISRTPEVTCVVVDVSHEDPEVKFNWYVDGVEVHNAKTKPREEQYNSTYRVVSVLTVLHQDWLNGKEYKCKVSNKALPAPIEKTISKAKGQPREPQVYTLPPSRDELTKNQVSLTCLVKGFYPSDIAVEWESNGQPENNYKTTPPVLDSDGSFFLYSKLTVDKSRWQQGNVFSCSVMHEALHNHYTQKSLSLSPGKGSSETQANSTTDALNVLLIIVDDLRPSLGCYGDKLVRSPNIDQLASHSLLFQNAFAQQAVCAPSRVSFLTGRRPDTTRLYDFNSYWRVHAGNFSTIPQYFKENGYVTMSVGKVFHPGISSNHTDDSPYSWSFPPYHPSSEKYENTKTCRGPDGELHANLLCPVDVLDVPEGTLPDKQSTEQAIQLLEKMKTSASPFFLAVGYHKPHIPFRYPKEFQKLYPLENITLAPDPEVPDGLPPVAYNPWMDIRQREDVQALNISVPYGPIPVDFQRKIRQSYFASVSYLDTQVGRLLSALDDLQLANSTIIAFTSDHGWALGEHGEWAKYSNFDVATHVPLIFYVPGRTASLPEAGEKLFPYLDPFDSASQLMEPGRQSMDLVELVSLFPTLAGLAGLQVPPRCPVPSFHVELCREGKNLLKHFRFRDLEEDPYLPGNPRELIAYSQYPRPSDIPQWNSDKPSLKDIKIMGYSIRTIDYRYTVWVGFNPDEFLANFSDIHAGELYFVDSDPLQDHNMYNDSQGGDLFQLLMP

SEQ ID NO: 14 - protein, 975 aa, Artificial Sequence
  Amino acid sequence of fusion protein of the heavy-chain of humanized anti-hTfR antibody No.3 and hI2S
EVQLVQSGAEVKKPGESLKISCKGSGYSFTNYWLGWVRQMPGKGLEWMGDIYPGGDYPTYSEKFKVQVTISADKSISTAYLQWSSLKASDTAMYYCARSGNYDEVAYWGQGTLVTVSSASTKGPSVFPLAPSSKSTSGGTAALGCLVKDYFPEPVTVSWNSGALTSGVHTFPAVLQSSGLYSLSSVVTVPSSSLGTQTYICNVNHKPSNTKVDKKVEPKSCDKTHTCPPCPAPELLGGPSVFLFPPKPKDTLMISRTPEVTCVVVDVSHEDPEVKFNWYVDGVEVHNAKTKPREEQYNSTYRVVSVLTVLHQDWLNGKEYKCKVSNKALPAPIEKTISKAKGQPREPQVYTLPPSRDELTKNQVSLTCLVKGFYPSDIAVEWESNGQPENNYKTTPPVLDSDGSFFLYSKLTVDKSRWQQGNVFSCSVMHEALHNHYTQKSLSLSPGKGSSETQANSTTDALNVLLIIVDDLRPSLGCYGDKLVRSPNIDQLASHSLLFQNAFAQQAVCAPSRVSFLTGRRPDTTRLYDFNSYWRVHAGNFSTIPQYFKENGYVTMSVGKVFHPGISSNHTDDSPYSWSFPPYHPSSEKYENTKTCRGPDGELHANLLCPVDVLDVPEGTLPDKQSTEQAIQLLEKMKTSASPFFLAVGYHKPHIPFRYPKEFQKLYPLENITLAPDPEVPDGLPPVAYNPWMDIRQREDVQALNISVPYGPIPVDFQRKIRQSYFASVSYLDTQVGRLLSALDDLQLANSTIIAFTSDHGWALGEHGEWAKYSNFDVATHVPLIFYVPGRTASLPEAGEKLFPYLDPFDSASQLMEPGRQSMDLVELVSLFPTLAGLAGLQVPPRCPVPSFHVELCREGKNLLKHFRFRDLEEDPYLPGNPRELIAYSQYPRPSDIPQWNSDKPSLKDIKIMGYSIRTIDYRYTVWVGFNPDEFLANFSDIHAGELYFVDSDPLQDHNMYNDSQGGDLFQLLMP

SEQ ID NO: 15 - protein, 107 aa, Artificial Sequence
  Amino acid sequence of the light-chain variable region of humanized anti-hTfR antibody No.1
DIQVTQSPSFLSASVGDRVTITCKASQDVNSAVAWFQQKPGKAPKLLIYWTSTRHTGVPDRFSGSGSGTVYTLTISSLQPEDFATYYCQQHYSTPRTFGGGTKVEIK

SEQ ID NO: 16 - protein, 116 aa, Artificial Sequence
  Amino acid sequence of the heavy-chain variable region of humanized anti-hTfR antibody No.1
EVQLVESGGGLVQPGGSLRLSCAASGLTFSNYGMSWVRQAPGKGLELVANINTNGGSTYYPDSVKGRFTISRDNAKNSLYLQMNSLRAEDTAVYYCTNNRYDEDYWGQGTLVTVSS

SEQ ID NO: 17 - protein, 107 aa, Artificial Sequence
  Amino acid sequence of the light-chain variable region of humanized anti-hTfR antibody No.2
EIVLTQSPDFQSVTPKEKVTITCRASQSISNNLQWYQQKPDQSPKLLIKYASQSISGIPSRFSGSGSGTDFTLTINSLEAEDAATYLCQQSNSWPRTFGQGTKVEIK

SEQ ID NO: 18 - protein, 120 aa, Artificial Sequence
  Amino acid sequence of the heavy-chain variable region of humanized anti-hTfR antibody No.2
QVQLVQSGAEVKKPGASVKVSCKASGYTFTDYVMHWVRQAPGQGLEWIGVISTYYGHGSYNQRFKGRATMTVDKSISTAYMELVRLRSDDTAVYYCVRGGYGSSSLAGNFDVWGQGTTVT

SEQ ID NO: 19 - protein, 112 aa, Artificial Sequence
  Amino acid sequence of the light-chain variable region of humanized anti-hTfR antibody No.3
DIVMTQTPLSLSVTPGQPASISCRSSQSLVHSNGNTYLHWYLQKPGQSPQLLIYKVSNRFSGVPDRFSGSGSGTDFTLKISRVEAEDVGVYYCSQSTHVPWTFGQGTKVEIK

SEQ ID NO: 20 - protein, 118 aa, Artificial Sequence
  Amino acid sequence of the heavy-chain variable region of humanized anti-hTfR antibody No.3
EVQLVQSGAEVKKPGESLKISCKGSGYSFTNYWLGWVRQMPGKGLEWMGDIYPGGDYPTYSEKFKVQVTISADKSISTAYLQWSSLKASDTAMYYCARSGNYDEVAYWGQGTLVTVSS

SEQ ID NO: 21 - DNA, 725 bp, Artificial Sequence
  Nucleotide seuquence encoding amino acid sequence of the light-chain of humanized anti-hTfR antibody No.1, synthetic sequence
acgcgtgccgccaccatgggctggagctggattctgctgttcctcctgagcgtgacagcaggagtgcacagcgacatccaggtcacacagtcaccaagttttctgagcgcaagcgtgggcgacagggtcactatcacatgcaaggcaagccaggacgtgaactccgcagtggcctggttccagcagaagccagggaaagcacccaagctgctgatctattggacctctacaaggcacaccggtgtcccagatcggttctcaggttccggcagcggaacagtgtatactctgaccatttccagcctgcagcctgaagacttcgctacttactattgccagcagcattactccaccccaagaacatttggcggagggactaaagtggagatcaagaggaccgtggccgctccctccgtcttcatttttccccctagcgacgaacagctgaagagtggcacagcctcagtggtctgtctgctgaacaatttctaccctagggaggctaaagtgcagtggaaggtcgataacgcactgcagtctggaaatagtcaggagtcagtgacagaacaggactccaaagatagcacttattctctgtctagtacactgactctgagcaaggccgattacgaaaagcacaaagtgtatgcttgcgaagtcacccatcaggggctgtcatcaccagtcaccaagtcattcaatagaggcgagtgctaagcggccgc

SEQ ID NO: 22 - protein, 725 aa, Artificial Sequence
  Nucleotide seuquence encoding amino acid sequence of the light-chain of humanized anti-hTfR antibody No.2, synthetic sequence
ACGCGTGCCGCCACCATGGGCTGGAGCTGGATTCTGCTGTTCCTCCTGAGCGTGACAGCAGGAGTGCACAGCGAAATTGTGCTGACCCAGTCTCCCGATTTCCAGTCCGTGACCCCCAAGGAGAAAGTCACCATCACATGCAGAGCATCACAGTCCATTAGCAACAATCTGCAGTGGTACCAGCAGAAGCCAGACCAGAGCCCCAAGCTGCTGATCAAATATGCCTCTCAGAGTATTTCAGGCATACCTTCTAGGTTCTCCGGTAGCGGCTCTGGAACCGACTTTACTCTGACCATCAACAGTCTGGAGGCTGAAGATGCCGCTACATACTTGTGCCAGCAGAGTAATTCATGGCCTAGGACCTTTGGCCAGGGGACAAAGGTGGAGATCAAAAGGACTGTGGCAGCCCCAAGTGTCTTCATTTTTCCCCCTTCAGACGAACAGCTGAAGAGCGGCACAGCATCTGTGGTCTGTCTGCTGAACAATTTCTACCCACGGGAGGCTAAGGTGCAGTGGAAAGTCGATAACGCACTGCAGTCCGGAAATAGCCAGGAGTCTGTGACTGAACAGGACAGTAAGGATTCAACCTATTCCCTGTCCAGCACACTGACTCTGAGCAAAGCCGATTACGAGAAGCACAAAGTGTATGCTTGCGAAGTCACACATCAGGGGCTGTCTAGTCCCGTGACTAAGTCTTTTAATAGGGGTGAATGTTAAGCGGCCGC

SEQ ID NO: 23 - DNA, 740 bp, Artificial Sequence
  Nucleotide seuquence encoding amino acid sequence of the light-chain of humanized anti-hTfR antibody No.3, synthetic sequence
acgcgtgccgccaccatgggctggagctggattctgctgttcctcctgagcgtgacagcaggagtgcacagcgacatcgtgatgacccagactcccctgagcctgagcgtgacacctggccagcctgccagcatcagctgcagaagctctcagagcctggtgcacagcaacggcaacacctacctgcactggtatctgcagaagcccggccagagccctcagctgctgatctacaaggtgtccaacagattcagcggcgtgcccgacagattctccggcagcggctctggcaccgacttcaccctgaagatttccagagtggaagccgaggacgtgggcgtgtactactgcagccagagcacccacgtgccctggacattcggccagggcaccaaggtggaaatcaagagaaccgtggccgctcccagcgtgttcatcttcccacctagcgacgagcagctgaagtccggcacagcctctgtcgtgtgcctgctgaacaacttctacccccgcgaggccaaggtgcagtggaaggtggacaacgccctgcagagcggcaacagccaggaaagcgtgaccgagcaggactccaaggacagcacctacagcctgagcagcaccctgaccctgagcaaggccgactacgagaagcacaaggtgtacgcctgcgaagtgacccaccagggcctgtctagccccgtgaccaagagcttcaacagaggcgagtgctaagcggccgc

SEQ ID NO: 24 - DNA, 3002 bp, Artificial Sequence
  Nucleotide seuquence encoding amino acid sequence of fusion protein of the heavy-chain of humanized anti-hTfR antibody No.1 and hI2S, synthetic sequence
acgcgtgccgccaccatgggctggagctggattctgctgttcctcctgagcgtgacagcaggagtgcacagcgaagtgcagctggtcgaatcagggggggggctggtgcagcctggaggcagcctgagactgtcctgcgccgcttctggcttgacctttagcaactacgggatgtcctgggtgcggcaggctcctggcaagggactggagttggtggccaacatcaataccaacggcggaagtacatactatcccgattcagtgaagggccggttcaccatcagcagggacaacgccaagaacagcctgtatctgcagatgaactctctgagggccgaggatacagccgtgtactattgcactaacaaccggtacgacgaggactattggggccagggcaccctggtgacagtgtctagcgcctctaccaagggcccaagcgtgtttcctctggctccatcctctaaatccacctctggcggcacagccgctctgggctgtctggtgaaggattacttcccagagcccgtgacagtgtcttggaacagcggcgccctgacctccggcgtgcacacatttcctgctgtgctgcagagctccggcctgtacagcctgtctagcgtggtgaccgtgccatcctctagcctgggcacccagacatatatctgcaacgtgaatcacaagcccagcaatacaaaggtggataagaaggtggagccaaagtcctgtgacaagacccacacatgccccccttgtcctgctccagagctgctgggaggaccaagcgtgttcctgtttccacccaagcccaaggataccctgatgatctctcggaccccagaggtgacatgcgtggtggtggatgtgagccacgaggaccccgaggtgaagttcaactggtatgtggacggcgtggaggtgcacaatgctaagaccaagcccagggaggagcagtacaactccacctatagagtggtgtctgtgctgacagtgctgcaccaggattggctgaacggcaaggagtataagtgcaaggtgtccaataaggccctgcccgctcctatcgagaagaccatctctaaggccaagggccagcccagagagcctcaggtgtacacactgcctccatcccgggatgagctgaccaagaaccaggtgtctctgacatgtctggtcaagggcttctatccctctgacatcgccgtggagtgggagagcaatggccagcctgagaacaattacaagaccacaccccctgtgctggattccgacggctctttctttctgtatagcaagctgaccgtggacaagtcccggtggcagcagggcaacgtgttcagctgttccgtgatgcacgaagctctgcataatcactatactcagaaatccctgtcactgtcacctggtaaaggatcttccgaaacgcaggccaactcgaccacagatgctctgaacgttcttctcatcatcgtggatgacctgcgcccctccctgggctgttatggggataagctggtgaggtccccaaatattgaccaactggcatcccacagcctcctcttccagaatgcctttgcgcagcaagcagtgtgcgccccgagccgcgtttctttcctcactggcaggagacctgacaccacccgcctgtacgacttcaactcctactggagggtgcacgctggaaacttctccaccatcccccagtacttcaaggagaatggctatgtgaccatgtcggtgggaaaagtctttcaccctgggatatcttctaaccataccgatgattctccgtatagctggtcttttccaccttatcatccttcctctgagaagtatgaaaacactaagacatgtcgagggccagatggagaactccatgccaacctgctttgccctgtggatgtgctggatgttcccgagggcaccttgcctgacaaacagagcactgagcaagccatacagttgttggaaaagatgaaaacgtcagccagtcctttcttcctggccgttgggtatcataagccacacatccccttcagataccccaaggaatttcagaagttgtatcccttggagaacatcaccctggcccccgatcccgaggtccctgatggcctaccccctgtggcctacaacccctggatggacatcaggcaacgggaagacgtccaagccttaaacatcagtgtgccgtatggtccaattcctgtggactttcagcggaaaatccgccagagctactttgcctctgtgtcatatttggatacacaggtcggccgcctcttgagtgctttggacgatcttcagctggccaacagcaccatcattgcatttacctcggatcatgggtgggctctaggtgaacatggagaatgggccaaatacagcaattttgatgttgctacccatgttcccctgatattctatgttcctggaaggacggcttcacttccggaggcaggcgagaagcttttcccttacctcgacccttttgattccgcctcacagttgatggagccaggcaggcaatccatggaccttgtggaacttgtgtctctttttcccacgctggctggacttgcaggactgcaggttccacctcgctgccccgttccttcatttcacgttgagctgtgcagagaaggcaagaaccttctgaagcattttcgattccgtgacttggaagaagatccgtacctccctggtaatccccgtgaactgattgcctatagccagtatccccggccttcagacatccctcagtggaattctgacaagccgagtttaaaagatataaagatcatgggctattccatacgcaccatagactataggtatactgtgtgggttggcttcaatcctgatgaatttctagctaacttttctgacatccatgcaggggaactgtattttgtggattctgacccattgcaggatcacaatatgtataatgattcccaaggtggagaccttttccagttgttgatgccttaagcggccgc

SEQ ID NO: 25 - DNA, 3023 bp, Artificial Sequence
  Nucleotide seuquence encoding amino acid sequence of fusion protein of the heavy-chain of humanized anti-hTfR antibody No.2 and hI2S, synthetic sequence
acgcgtgccgccaccatgggctggagctggattctgctgttcctcctgagcgtgacagcaggagtgcacagccaggtgcagctggtccagtcaggagccgaagtgaaaaagcccggagcctcagtcaaagtgtcttgtaaagcatcaggttatacatttacagactacgtcatgcactgggtgaggcaggcacctggacagggtctggaatggatcggcgtgatctccacttactatggccatggaagctacaaccagagattcaagggcagggcgacaatgactgtagacaaatcaatttccactgcttatatggagctggtaaggctgcggtccgacgataccgctgtgtactattgcgtacgaggaggatacggctccagctctctggctggtaatttcgatgtgtgggggcagggtaccacagtcaccgtgagttcagcaagcacaaagggcccatctgtgtttccactggccccctccagcaaaagcacctctgggggtacagccgctctgggatgtctggtgaaggattatttcccagagccagtcaccgtgtcctggaacagcggagccctgacatctggagtccacacttttccagctgtgctgcagtctagtgggctgtactccctgtcatccgtggtcactgtccccagctctagtctgggtacccagacatatatctgcaacgtgaatcacaagccatctaataccaaagtcgacaagaaagtggaacccaagtcctgtgataaaactcatacctgccccccttgtcctgcaccagagctgctgggaggaccatccgtgttcctgtttccacccaagcctaaagacaccctgatgattagccgaactcccgaagtcacctgcgtggtcgtggacgtgtctcacgaggaccctgaagtcaagtttaactggtacgtggatggcgtcgaggtgcataatgctaagacaaaaccccgagaggaacagtacaacagtacatatcgtgtcgtgtcagtgctgaccgtcctgcatcaggactggctgaacgggaaggaatataagtgcaaagtgtccaataaggcactgcccgcccctatcgagaaaaccattagcaaggccaaaggacagcctagggaaccacaggtgtacacactgcctccatcccgggacgagctgactaagaaccaggtcagcctgacctgtctggtgaaaggcttctatccttcagatatcgctgtggagtgggaaagtaatggacagccagagaacaattacaagactaccccccctgtgctggactctgatgggagtttctttctgtattctaagctgaccgtggataaaagtcggtggcagcagggtaatgtctttagttgttcagtgatgcacgaagcactgcacaaccactacacccagaaatcactgtcactgtcaccagggaaaggatcttccgaaacgcaggccaactcgaccacagatgctctgaacgttcttctcatcatcgtggatgacctgcgcccctccctgggctgttatggggataagctggtgaggtccccaaatattgaccaactggcatcccacagcctcctcttccagaatgcctttgcgcagcaagcagtgtgcgccccgagccgcgtttctttcctcactggcaggagacctgacaccacccgcctgtacgacttcaactcctactggagggtgcacgctggaaacttctccaccatcccccagtacttcaaggagaatggctatgtgaccatgtcggtgggaaaagtctttcaccctgggatatcttctaaccataccgatgattctccgtatagctggtcttttccaccttatcatccttcctctgagaagtatgaaaacactaagacatgtcgagggccagatggagaactccatgccaacctgctttgccctgtggatgtgctggatgttcccgagggcaccttgcctgacaaacagagcactgagcaagccatacagttgttggaaaagatgaaaacgtcagccagtcctttcttcctggccgttgggtatcataagccacacatccccttcagataccccaaggaatttcagaagttgtatcccttggagaacatcaccctggcccccgatcccgaggtccctgatggcctaccccctgtggcctacaacccctggatggacatcaggcaacgggaagacgtccaagccttaaacatcagtgtgccgtatggtccaattcctgtggactttcagcggaaaatccgccagagctactttgcctctgtgtcatatttggatacacaggtcggccgcctcttgagtgctttggacgatcttcagctggccaacagcaccatcattgcatttacctcggatcatgggtgggctctaggtgaacatggagaatgggccaaatacagcaattttgatgttgctacccatgttcccctgatattctatgttcctggaaggacggcttcacttccggaggcaggcgagaagcttttcccttacctcgacccttttgattccgcctcacagttgatggagccaggcaggcaatccatggaccttgtggaacttgtgtctctttttcccacgctggctggacttgcaggactgcaggttccacctcgctgccccgttccttcatttcacgttgagctgtgcagagaaggcaagaaccttctgaagcattttcgattccgtgacttggaagaagatccgtacctccctggtaatccccgtgaactgattgcctatagccagtatccccggccttcagacatccctcagtggaattctgacaagccgagtttaaaagatataaagatcatgggctattccatacgcaccatagactataggtatactgtgtgggttggcttcaatcctgatgaatttctagctaacttttctgacatccatgcaggggaactgtattttgtggattctgacccattgcaggatcacaatatgtataatgattcccaaggtggagaccttttccagttgttgatgccttaagcggccgc

SEQ ID NO: 26 - DNA, 3011 bp, Artificial Sequence
  Nucleotide seuquence encoding amino acid sequence of fusion protein of the heavy-chain of humanized anti-hTfR antibody No.3 and hI2S, synthetic sequence
acgcgtgccgccaccatgggctggagctggattctgctgttcctcctgagcgtgacagcaggagtgcacagcgaggtgcaactagtgcagtctggagcagaggtgaaaaagcccggggagtctctgaagatttcctgtaagggttctggatacagctttaccaactactggctgggatgggtgcgccagatgcccgggaaaggcctggagtggatgggggacatctaccccggcggagactaccctacatacagcgagaagttcaaggtccaggtcaccatctcagccgacaagtccatcagcaccgcctacctgcagtggagcagcctgaaggcctcggacaccgccatgtattactgtgcgagatcaggcaattacgacgaagtggcctactggggccaaggaaccctggtcaccgtctcctcagctagcaccaagggcccatcggtcttccccctggcaccctcctccaagagcacctctgggggcacagcggccctgggctgcctggtcaaggactacttccccgaaccggtgacggtgtcgtggaactcaggcgccctgaccagcggcgtgcacaccttcccggctgtcctacagtcctcaggactctactccctcagcagcgtggtgaccgtgccctccagcagcttgggcacccagacctacatctgcaacgtgaatcacaagcccagcaacaccaaggtggacaagaaagttgagcccaaatcttgtgacaaaactcacacgtgcccaccgtgcccagcacctgaactcctgggaggtccgtcagtcttcctcttccccccaaaacccaaggacaccctcatgatctcccggacccctgaggtcacatgcgtggtggtggacgtgagccacgaagaccctgaggtcaagttcaactggtacgtggacggcgtggaggtgcataatgccaagacaaagccgcgggaggagcagtacaacagcacgtaccgggtggtcagcgtcctcaccgtcctgcaccaggactggctgaatggcaaggagtacaagtgcaaggtctccaacaaagccctcccagcccccatcgagaaaaccatctccaaagccaaagggcagccccgagaaccacaggtgtacaccctgcccccatcccgggatgagctgaccaagaaccaggtcagcctgacctgcctggtcaaaggcttctatcccagcgacatcgccgtggagtgggagagcaatgggcagccggagaacaactacaagaccacgcctcccgtgctggactccgacggctccttcttcctctacagcaagctcaccgtggacaagagcaggtggcagcaggggaacgtcttctcatgctccgtgatgcatgaggctctgcacaaccactacacgcagaagagcctctccctgtctccgggtaaaggatcttccgaaacgcaggccaactcgaccacagatgctctgaacgttcttctcatcatcgtggatgacctgcgcccctccctgggctgttatggggataagctggtgaggtccccaaatattgaccaactggcatcccacagcctcctcttccagaatgcctttgcgcagcaagcagtgtgcgccccgagccgcgtttctttcctcactggcaggagacctgacaccacccgcctgtacgacttcaactcctactggagggtgcacgctggaaacttctccaccatcccccagtacttcaaggagaatggctatgtgaccatgtcggtgggaaaagtctttcaccctgggatatcttctaaccataccgatgattctccgtatagctggtcttttccaccttatcatccttcctctgagaagtatgaaaacactaagacatgtcgagggccagatggagaactccatgccaacctgctttgccctgtggatgtgctggatgttcccgagggcaccttgcctgacaaacagagcactgagcaagccatacagttgttggaaaagatgaaaacgtcagccagtcctttcttcctggccgttgggtatcataagccacacatccccttcagataccccaaggaatttcagaagttgtatcccttggagaacatcaccctggcccccgatcccgaggtccctgatggcctaccccctgtggcctacaacccctggatggacatcaggcaacgggaagacgtccaagccttaaacatcagtgtgccgtatggtccaattcctgtggactttcagcggaaaatccgccagagctactttgcctctgtgtcatatttggatacacaggtcggccgcctcttgagtgctttggacgatcttcagctggccaacagcaccatcattgcatttacctcggatcatgggtgggctctaggtgaacatggagaatgggccaaatacagcaattttgatgttgctacccatgttcccctgatattctatgttcctggaaggacggcttcacttccggaggcaggcgagaagcttttcccttacctcgacccttttgattccgcctcacagttgatggagccaggcaggcaatccatggaccttgtggaacttgtgtctctttttcccacgctggctggacttgcaggactgcaggttccacctcgctgccccgttccttcatttcacgttgagctgtgcagagaaggcaagaaccttctgaagcattttcgattccgtgacttggaagaagatccgtacctccctggtaatccccgtgaactgattgcctatagccagtatccccggccttcagacatccctcagtggaattctgacaagccgagtttaaaagatataaagatcatgggctattccatacgcaccatagactataggtatactgtgtgggttggcttcaatcctgatgaatttctagctaacttttctgacatccatgcaggggaactgtattttgtggattctgacccattgcaggatcacaatatgtataatgattcccaaggtggagaccttttccagttgttgatgccttaataagcggccgc

SEQ ID NO: 27 - DNA, 20 bp, Artificial Sequence
  Primer Hyg-Sfi5', synthetic sequence
gaggccgcctcggcctctga

SEQ ID NO: 28 - DNA, 29 bp, Artificial Sequence
  Primer Hyg-BstX3', synthetic sequence
aaccatcgtgatgggtgctattcctttgc